European Patent Application EP 4 159 907 A1, published April 5, 2023. Title: A Nonwoven Fabrics and a Method for Manufacturing thereof. Applicant: Spiber Inc. Shinwa corp. The sequence listing filed with the application follows.

SEQUENCE LISTING (44 sequences)

SEQ ID NO: 1 - protein, 50 aa, Araneus diadematus
SGCDVLVQALLEVVSALVSILGSSSIGQINYGASAQYTQMVGQSVAQALA

SEQ ID NO: 2 - protein, 30 aa, Araneus diadematus
SGCDVLVQALLEVVSALVSILGSSSIGQIN

SEQ ID NO: 3 - protein, 21 aa, Araneus diadematus
SGCDVLVQALLEVVSALVSIL

SEQ ID NO: 4 - protein, 1154 aa, Artificial Sequence
  recombinant spider silk protein ADF3KaiLargeNRSH1
MHHHHHHHHHHSSGSSLEVLFQGPARAGSGQQGPGQQGPGQQGPGQQGPYGPGASAAAAAAGGYGPGSGQQGPSQQGPGQQGPGGQGPYGPGASAAAAAAGGYGPGSGQQGPGGQGPYGPGSSAAAAAAGGNGPGSGQQGAGQQGPGQQGPGASAAAAAAGGYGPGSGQQGPGQQGPGGQGPYGPGASAAAAAAGGYGPGSGQGPGQQGPGGQGPYGPGASAAAAAAGGYGPGSGQQGPGQQGPGQQGPGGQGPYGPGASAAAAAAGGYGPGYGQQGPGQQGPGGQGPYGPGASAASAASGGYGPGSGQQGPGQQGPGGQGPYGPGASAAAAAAGGYGPGSGQQGPGQQGPGQQGPGQQGPGGQGPYGPGASAAAAAAGGYGPGSGQQGPGQQGPGQQGPGQQGPGQQGPGQQGPGQQGPGQQGPGQQGPGGQGAYGPGASAAAGAAGGYGPGSGQQGPGQQGPGQQGPGQQGPGQQGPGQQGPGQQGPGQQGPYGPGASAAAAAAGGYGPGSGQQGPGQQGPGQQGPGGQGPYGPGAASAAVSVSRARAGSGQQGPGQQGPGQQGPGQQGPYGPGASAAAAAAGGYGPGSGQQGPSQQGPGQQGPGGQGPYGPGASAAAAAAGGYGPGSGQQGPGGQGPYGPGSSAAAAAAGGNGPGSGQQGAGQQGPGQQGPGASAAAAAAGGYGPGSGQQGPGQQGPGGQGPYGPGASAAAAAAGGYGPGSGQGPGQQGPGGQGPYGPGASAAAAAAGGYGPGSGQQGPGQQGPGQQGPGGQGPYGPGASAAAAAAGGYGPGYGQQGPGQQGPGGQGPYGPGASAASAASGGYGPGSGQQGPGQQGPGGQGPYGPGASAAAAAAGGYGPGSGQQGPGQQGPGQQGPGQQGPGGQGPYGPGASAAAAAAGGYGPGSGQQGPGQQGPGQQGPGQQGPGQQGPGQQGPGQQGPGQQGPGQQGPGGQGAYGPGASAAAGAAGGYGPGSGQQGPGQQGPGQQGPGQQGPGQQGPGQQGPGQQGPGQQGPYGPGASAAAAAAGGYGPGSGQQGPGQQGPGQQGPGGQGPYGPGAASAAVSVGGYGPQSSSVPVASAVASRLSSPAASSRVSSAVSSLVSSGPTKHAALSNTISSVVSQVSASNPGLSGCDVLVQALLEVVSALVSIL

SEQ ID NO: 5 - protein, 24 aa, Artificial Sequence
  His tag and start codon
MHHHHHHHHHHSSGSSLEVLFQGP

SEQ ID NO: 6 - protein, 597 aa, Artificial Sequence
  Met-PRT380
MGPGQQGPYGPGASAAAAAGQNGPGSGQQGPGQSAAAAAGQYGPGQQGPGQQGPGSSAAAAAGPGQYGPGQQGPSASAAAAAGPGSGQQGPGASAAAAAGQYGPGQQGPGQQGPGSSAAAAAGQYGSGPGQQGPYGSAAAAAGPGSGQYGQGPYGPGASAAAAAGPGQYGPGQQGPSASAAAAAGSGQQGPGQYGPYASAAAAAGQYGSGPGQQGPYGPGQSAAAAAGSGQQGPGQQGPYASAAAAAGPGQQGPYGPGSSAAAAAGQYGYGPGQQGPYGPGASAAAAAGQNGPGSGQYGPGQQGPGQSAAAAAGPGQQGPYGPGASAAAAAGQYGPGQQGPGQYGPGSSAAAAAGPGQQGPYGPGSSAAAAAGQYGPGQQGPYGPGQSAAAAAGQYQQGPGQQGPYGPGASAAAAAGPGQQGPYGPGASAAAAAGPGQYGPGQQGPSASAAAAAGQYGSGPGQYGPYGPGQSAAAAAGPGSGQQGQGPYGPGASAAAAAGQYGPGQQGPYGPGQSAAAAAGPGSGQYGPGASAAAAAGQNGPGSGQYGPGQQGPGQSAAAAAGQYQQGPGQQGPYGPGASAAAAAGPGSGQQGPGAS

SEQ ID NO: 7 - protein, 590 aa, Artificial Sequence
  Met-PRT410
MGPGQQGPYGPGASAAAAAGQNGPGSGQQGPGQSGQYGPGQQGPGQQGPGSSAAAAAGPGQYGPGQQGPSASAAAAAGPGSGQQGPGASGQYGPGQQGPGQQGPGSSAAAAAGQYGSGPGQQGPYGSAAAAAGPGSGQYGQGPYGPGASGPGQYGPGQQGPSASAAAAAGSGQQGPGQYGPYASAAAAAGQYGSGPGQQGPYGPGQSGSGQQGPGQQGPYASAAAAAGPGQQGPYGPGSSAAAAAGQYGYGPGQQGPYGPGASGQNGPGSGQYGPGQQGPGQSAAAAAGPGQQGPYGPGASAAAAAGQYGPGQQGPGQYGPGSSGPGQQGPYGPGSSAAAAAGQYGPGQQGPYGPGQSAAAAAGQYQQGPGQQGPYGPGASGPGQQGPYGPGASAAAAAGPGQYGPGQQGPSASAAAAAGQYGSGPGQYGPYGPGQSGPGSGQQGQGPYGPGASAAAAAGQYGPGQQGPYGPGQSAAAAAGPGSGQYGPGASGQNGPGSGQYGPGQQGPGQSAAAAAGQYQQGPGQQGPYGPGASAAAAAGQYGSGPGQQGPYGPGQSGSGQQGPGQQGPYASAAAAAGPGSGQQGPGAS

SEQ ID NO: 8 - protein, 565 aa, Artificial Sequence
  Met-PRT525
MGPGQQGPYGPGASAAAAAAAGSNGPGSGQQGPGQSGQYGPGQQGPGQQGPGSSAAAAAAAGPGQYGPGQQGPSASAAAAAAAGPGSGQQGPGASGQYGPGQQGPGQQGPGSSAAAAAAAGSYGSGPGQQGPYGSAAAAAAAGPGSGQYGQGPYGPGASGPGQYGPGQQGPSASAAAAAAAGSGQQGPGQYGPYASAAAAAAAGSYGSGPGQQGPYGPGQSGSGQQGPGQQGPYASAAAAAAAGPGQQGPYGPGSSAAAAAAAGSYGYGPGQQGPYGPGASGQNGPGSGQYGPGQQGPGPSAAAAAAAGPGQQGPYGPGASAAAAAAAGSYGPGQQGPGQYGPGSSGPGQQGPYGPGSSAAAAAAAGSYGPGQQGPYGPGPSAAAAAAAGSYQQGPGQQGPYGPGASGPGQQGPYGPGASAAAAAAAGPGQYGPGQQGPSASAAAAAAAGSYGSGPGQYGPYGPGQSGPGSGQQGQGPYGPGASAAAAAAAGSYGPGQQGPYGPGPSAAAAAAAGPGSGQYGPGASGQNGPGSGQYGPGQQGPGPSAAAAAAAGPGSGQQGPGAS

SEQ ID NO: 9 - protein, 2364 aa, Artificial Sequence
  Met-PRT799
MGPGQQGPYGPGASAAAAAGQNGPGSGQQGPGQSGQYGPGQQGPGQQGPGSSAAAAAGPGQYGPGQQGPSASAAAAAGPGSGQQGPGASGQYGPGQQGPGQQGPGSSAAAAAGQYGSGPGQQGPYGSAAAAAGPGSGQYGQGPYGPGASGPGQYGPGQQGPSASAAAAAGSGQQGPGQYGPYASAAAAAGQYGSGPGQQGPYGPGQSGSGQQGPGQQGPYASAAAAAGPGQQGPYGPGSSAAAAAGQYGYGPGQQGPYGPGASGQNGPGSGQYGPGQQGPGQSAAAAAGPGQQGPYGPGASAAAAAGQYGPGQQGPGQYGPGSSGPGQQGPYGPGSSAAAAAGQYGPGQQGPYGPGQSAAAAAGQYQQGPGQQGPYGPGASGPGQQGPYGPGASAAAAAGPGQYGPGQQGPSASAAAAAGQYGSGPGQYGPYGPGQSGPGSGQQGQGPYGPGASAAAAAGQYGPGQQGPYGPGQSAAAAAGPGSGQYGPGASGQNGPGSGQYGPGQQGPGQSAAAAAGQYQQGPGQQGPYGPGASAAAAAGQYGSGPGQQGPYGPGQSGSGQQGPGQQGPYASAAAAAGPGSGQQGPGASGQQGPYGPGASAAAAAGQNGPGSGQQGPGQSGQYGPGQQGPGQQGPGSSAAAAAGPGQYGPGQQGPSASAAAAAGPGSGQQGPGASGQYGPGQQGPGQQGPGSSAAAAAGQYGSGPGQQGPYGSAAAAAGPGSGQYGQGPYGPGASGPGQYGPGQQGPSASAAAAAGSGQQGPGQYGPYASAAAAAGQYGSGPGQQGPYGPGQSGSGQQGPGQQGPYASAAAAAGPGQQGPYGPGSSAAAAAGQYGYGPGQQGPYGPGASGQNGPGSGQYGPGQQGPGQSAAAAAGPGQQGPYGPGASAAAAAGQYGPGQQGPGQYGPGSSGPGQQGPYGPGSSAAAAAGQYGPGQQGPYGPGQSAAAAAGQYQQGPGQQGPYGPGASGPGQQGPYGPGASAAAAAGPGQYGPGQQGPSASAAAAAGQYGSGPGQYGPYGPGQSGPGSGQQGQGPYGPGASAAAAAGQYGPGQQGPYGPGQSAAAAAGPGSGQYGPGASGQNGPGSGQYGPGQQGPGQSAAAAAGQYQQGPGQQGPYGPGASAAAAAGQYGSGPGQQGPYGPGQSGSGQQGPGQQGPYASAAAAAGPGSGQQGPGASGQQGPYGPGASAAAAAGQNGPGSGQQGPGQSGQYGPGQQGPGQQGPGSSAAAAAGPGQYGPGQQGPSASAAAAAGPGSGQQGPGASGQYGPGQQGPGQQGPGSSAAAAAGQYGSGPGQQGPYGSAAAAAGPGSGQYGQGPYGPGASGPGQYGPGQQGPSASAAAAAGSGQQGPGQYGPYASAAAAAGQYGSGPGQQGPYGPGQSGSGQQGPGQQGPYASAAAAAGPGQQGPYGPGSSAAAAAGQYGYGPGQQGPYGPGASGQNGPGSGQYGPGQQGPGQSAAAAAGPGQQGPYGPGASAAAAAGQYGPGQQGPGQYGPGSSGPGQQGPYGPGSSAAAAAGQYGPGQQGPYGPGQSAAAAAGQYQQGPGQQGPYGPGASGPGQQGPYGPGASAAAAAGPGQYGPGQQGPSASAAAAAGQYGSGPGQYGPYGPGQSGPGSGQQGQGPYGPGASAAAAAGQYGPGQQGPYGPGQSAAAAAGPGSGQYGPGASGQNGPGSGQYGPGQQGPGQSAAAAAGQYQQGPGQQGPYGPGASAAAAAGQYGSGPGQQGPYGPGQSGSGQQGPGQQGPYASAAAAAGPGSGQQGPGASGQQGPYGPGASAAAAAGQNGPGSGQQGPGQSGQYGPGQQGPGQQGPGSSAAAAAGPGQYGPGQQGPSASAAAAAGPGSGQQGPGASGQYGPGQQGPGQQGPGSSAAAAAGQYGSGPGQQGPYGSAAAAAGPGSGQYGQGPYGPGASGPGQYGPGQQGPSASAAAAAGSGQQGPGQYGPYASAAAAAGQYGSGPGQQGPYGPGQSGSGQQGPGQQGPYASAAAAAGPGQQGPYGPGSSAAAAAGQYGYGPGQQGPYGPGASGQNGPGSGQYGPGQQGPGQSAAAAAGPGQQGPYGPGASAAAAAGQYGPGQQGPGQYGPGSSGPGQQGPYGPGSSAAAAAGQYGPGQQGPYGPGQSAAAAAGQYQQGPGQQGPYGPGASGPGQQGPYGPGASAAAAAGPGQYGPGQQGPSASAAAAAGQYGSGPGQYGPYGPGQSGPGSGQQGQGPYGPGASAAAAAGQYGPGQQGPYGPGQSAAAAAGPGSGQYGPGASGQNGPGSGQYGPGQQGPGQSAAAAAGQYQQGPGQQGPYGPGASAAAAAGQYGSGPGQQGPYGPGQSGSGQQGPGQQGPYASAAAAAGPGSGQQGSSVDKLAAALEHHHHHH

SEQ ID NO: 10 - protein, 597 aa, Artificial Sequence
  Met-PRT313
MGPGGQGPYGPGASAAAAAGGNGPGSGQQGPGGSAAAAAGGYGPGGQGPGQQGPGSSAAAAAGPGGYGPGGQGPSASAAAAAGPGSGQQGPGASAAAAAGGYGPGGQGPGQQGPGSSAAAAAGGYGSGPGQQGPYGSAAAAAGPGSGGYGQGPYGPGASAAAAAGPGGYGPGGQGPSASAAAAAGSGQQGPGGYGPYASAAAAAGGYGSGPGQQGPYGPGGSAAAAAGSGQQGPGQQGPYASAAAAAGPGGQGPYGPGSSAAAAAGGYGYGPGGQGPYGPGASAAAAAGGNGPGSGGYGPGQQGPGGSAAAAAGPGGQGPYGPGASAAAAAGGYGPGGQGPGGYGPGSSAAAAAGPGGQGPYGPGSSAAAAAGGYGPGQQGPYGPGGSAAAAAGGYQQGPGGQGPYGPGASAAAAAGPGGQGPYGPGASAAAAAGPGGYGPGGQGPSASAAAAAGGYGSGPGGYGPYGPGGSAAAAAGPGSGQQGQGPYGPGASAAAAAGGYGPGQQGPYGPGGSAAAAAGPGSGGYGPGASAAAAAGGNGPGSGGYGPGQQGPGGSAAAAAGGYQQGPGGQGPYGPGASAAAAAGPGSGQQGPGAS

SEQ ID NO: 11 - protein, 12 aa, Artificial Sequence
  HisTag
MHHHHHHSSGSS

SEQ ID NO: 12 - protein, 608 aa, Artificial Sequence
  PRT380
MHHHHHHSSGSSGPGQQGPYGPGASAAAAAGQNGPGSGQQGPGQSAAAAAGQYGPGQQGPGQQGPGSSAAAAAGPGQYGPGQQGPSASAAAAAGPGSGQQGPGASAAAAAGQYGPGQQGPGQQGPGSSAAAAAGQYGSGPGQQGPYGSAAAAAGPGSGQYGQGPYGPGASAAAAAGPGQYGPGQQGPSASAAAAAGSGQQGPGQYGPYASAAAAAGQYGSGPGQQGPYGPGQSAAAAAGSGQQGPGQQGPYASAAAAAGPGQQGPYGPGSSAAAAAGQYGYGPGQQGPYGPGASAAAAAGQNGPGSGQYGPGQQGPGQSAAAAAGPGQQGPYGPGASAAAAAGQYGPGQQGPGQYGPGSSAAAAAGPGQQGPYGPGSSAAAAAGQYGPGQQGPYGPGQSAAAAAGQYQQGPGQQGPYGPGASAAAAAGPGQQGPYGPGASAAAAAGPGQYGPGQQGPSASAAAAAGQYGSGPGQYGPYGPGQSAAAAAGPGSGQQGQGPYGPGASAAAAAGQYGPGQQGPYGPGQSAAAAAGPGSGQYGPGASAAAAAGQNGPGSGQYGPGQQGPGQSAAAAAGQYQQGPGQQGPYGPGASAAAAAGPGSGQQGPGAS

SEQ ID NO: 13 - protein, 601 aa, Artificial Sequence
  PRT410
MHHHHHHSSGSSGPGQQGPYGPGASAAAAAGQNGPGSGQQGPGQSGQYGPGQQGPGQQGPGSSAAAAAGPGQYGPGQQGPSASAAAAAGPGSGQQGPGASGQYGPGQQGPGQQGPGSSAAAAAGQYGSGPGQQGPYGSAAAAAGPGSGQYGQGPYGPGASGPGQYGPGQQGPSASAAAAAGSGQQGPGQYGPYASAAAAAGQYGSGPGQQGPYGPGQSGSGQQGPGQQGPYASAAAAAGPGQQGPYGPGSSAAAAAGQYGYGPGQQGPYGPGASGQNGPGSGQYGPGQQGPGQSAAAAAGPGQQGPYGPGASAAAAAGQYGPGQQGPGQYGPGSSGPGQQGPYGPGSSAAAAAGQYGPGQQGPYGPGQSAAAAAGQYQQGPGQQGPYGPGASGPGQQGPYGPGASAAAAAGPGQYGPGQQGPSASAAAAAGQYGSGPGQYGPYGPGQSGPGSGQQGQGPYGPGASAAAAAGQYGPGQQGPYGPGQSAAAAAGPGSGQYGPGASGQNGPGSGQYGPGQQGPGQSAAAAAGQYQQGPGQQGPYGPGASAAAAAGQYGSGPGQQGPYGPGQSGSGQQGPGQQGPYASAAAAAGPGSGQQGPGAS

SEQ ID NO: 14 - protein, 576 aa, Artificial Sequence
  PRT525
MHHHHHHSSGSSGPGQQGPYGPGASAAAAAAAGSNGPGSGQQGPGQSGQYGPGQQGPGQQGPGSSAAAAAAAGPGQYGPGQQGPSASAAAAAAAGPGSGQQGPGASGQYGPGQQGPGQQGPGSSAAAAAAAGSYGSGPGQQGPYGSAAAAAAAGPGSGQYGQGPYGPGASGPGQYGPGQQGPSASAAAAAAAGSGQQGPGQYGPYASAAAAAAAGSYGSGPGQQGPYGPGQSGSGQQGPGQQGPYASAAAAAAAGPGQQGPYGPGSSAAAAAAAGSYGYGPGQQGPYGPGASGQNGPGSGQYGPGQQGPGPSAAAAAAAGPGQQGPYGPGASAAAAAAAGSYGPGQQGPGQYGPGSSGPGQQGPYGPGSSAAAAAAAGSYGPGQQGPYGPGPSAAAAAAAGSYQQGPGQQGPYGPGASGPGQQGPYGPGASAAAAAAAGPGQYGPGQQGPSASAAAAAAAGSYGSGPGQYGPYGPGQSGPGSGQQGQGPYGPGASAAAAAAAGSYGPGQQGPYGPGPSAAAAAAAGPGSGQYGPGASGQNGPGSGQYGPGQQGPGPSAAAAAAAGPGSGQQGPGAS

SEQ ID NO: 15 - protein, 2375 aa, Artificial Sequence
  PRT799
MHHHHHHSSGSSGPGQQGPYGPGASAAAAAGQNGPGSGQQGPGQSGQYGPGQQGPGQQGPGSSAAAAAGPGQYGPGQQGPSASAAAAAGPGSGQQGPGASGQYGPGQQGPGQQGPGSSAAAAAGQYGSGPGQQGPYGSAAAAAGPGSGQYGQGPYGPGASGPGQYGPGQQGPSASAAAAAGSGQQGPGQYGPYASAAAAAGQYGSGPGQQGPYGPGQSGSGQQGPGQQGPYASAAAAAGPGQQGPYGPGSSAAAAAGQYGYGPGQQGPYGPGASGQNGPGSGQYGPGQQGPGQSAAAAAGPGQQGPYGPGASAAAAAGQYGPGQQGPGQYGPGSSGPGQQGPYGPGSSAAAAAGQYGPGQQGPYGPGQSAAAAAGQYQQGPGQQGPYGPGASGPGQQGPYGPGASAAAAAGPGQYGPGQQGPSASAAAAAGQYGSGPGQYGPYGPGQSGPGSGQQGQGPYGPGASAAAAAGQYGPGQQGPYGPGQSAAAAAGPGSGQYGPGASGQNGPGSGQYGPGQQGPGQSAAAAAGQYQQGPGQQGPYGPGASAAAAAGQYGSGPGQQGPYGPGQSGSGQQGPGQQGPYASAAAAAGPGSGQQGPGASGQQGPYGPGASAAAAAGQNGPGSGQQGPGQSGQYGPGQQGPGQQGPGSSAAAAAGPGQYGPGQQGPSASAAAAAGPGSGQQGPGASGQYGPGQQGPGQQGPGSSAAAAAGQYGSGPGQQGPYGSAAAAAGPGSGQYGQGPYGPGASGPGQYGPGQQGPSASAAAAAGSGQQGPGQYGPYASAAAAAGQYGSGPGQQGPYGPGQSGSGQQGPGQQGPYASAAAAAGPGQQGPYGPGSSAAAAAGQYGYGPGQQGPYGPGASGQNGPGSGQYGPGQQGPGQSAAAAAGPGQQGPYGPGASAAAAAGQYGPGQQGPGQYGPGSSGPGQQGPYGPGSSAAAAAGQYGPGQQGPYGPGQSAAAAAGQYQQGPGQQGPYGPGASGPGQQGPYGPGASAAAAAGPGQYGPGQQGPSASAAAAAGQYGSGPGQYGPYGPGQSGPGSGQQGQGPYGPGASAAAAAGQYGPGQQGPYGPGQSAAAAAGPGSGQYGPGASGQNGPGSGQYGPGQQGPGQSAAAAAGQYQQGPGQQGPYGPGASAAAAAGQYGSGPGQQGPYGPGQSGSGQQGPGQQGPYASAAAAAGPGSGQQGPGASGQQGPYGPGASAAAAAGQNGPGSGQQGPGQSGQYGPGQQGPGQQGPGSSAAAAAGPGQYGPGQQGPSASAAAAAGPGSGQQGPGASGQYGPGQQGPGQQGPGSSAAAAAGQYGSGPGQQGPYGSAAAAAGPGSGQYGQGPYGPGASGPGQYGPGQQGPSASAAAAAGSGQQGPGQYGPYASAAAAAGQYGSGPGQQGPYGPGQSGSGQQGPGQQGPYASAAAAAGPGQQGPYGPGSSAAAAAGQYGYGPGQQGPYGPGASGQNGPGSGQYGPGQQGPGQSAAAAAGPGQQGPYGPGASAAAAAGQYGPGQQGPGQYGPGSSGPGQQGPYGPGSSAAAAAGQYGPGQQGPYGPGQSAAAAAGQYQQGPGQQGPYGPGASGPGQQGPYGPGASAAAAAGPGQYGPGQQGPSASAAAAAGQYGSGPGQYGPYGPGQSGPGSGQQGQGPYGPGASAAAAAGQYGPGQQGPYGPGQSAAAAAGPGSGQYGPGASGQNGPGSGQYGPGQQGPGQSAAAAAGQYQQGPGQQGPYGPGASAAAAAGQYGSGPGQQGPYGPGQSGSGQQGPGQQGPYASAAAAAGPGSGQQGPGASGQQGPYGPGASAAAAAGQNGPGSGQQGPGQSGQYGPGQQGPGQQGPGSSAAAAAGPGQYGPGQQGPSASAAAAAGPGSGQQGPGASGQYGPGQQGPGQQGPGSSAAAAAGQYGSGPGQQGPYGSAAAAAGPGSGQYGQGPYGPGASGPGQYGPGQQGPSASAAAAAGSGQQGPGQYGPYASAAAAAGQYGSGPGQQGPYGPGQSGSGQQGPGQQGPYASAAAAAGPGQQGPYGPGSSAAAAAGQYGYGPGQQGPYGPGASGQNGPGSGQYGPGQQGPGQSAAAAAGPGQQGPYGPGASAAAAAGQYGPGQQGPGQYGPGSSGPGQQGPYGPGSSAAAAAGQYGPGQQGPYGPGQSAAAAAGQYQQGPGQQGPYGPGASGPGQQGPYGPGASAAAAAGPGQYGPGQQGPSASAAAAAGQYGSGPGQYGPYGPGQSGPGSGQQGQGPYGPGASAAAAAGQYGPGQQGPYGPGQSAAAAAGPGSGQYGPGASGQNGPGSGQYGPGQQGPGQSAAAAAGQYQQGPGQQGPYGPGASAAAAAGQYGSGPGQQGPYGPGQSGSGQQGPGQQGPYASAAAAAGPGSGQQGSSVDKLAAALEHHHHHH

SEQ ID NO: 16 - protein, 608 aa, Artificial Sequence
  PRT313
MHHHHHHSSGSSGPGGQGPYGPGASAAAAAGGNGPGSGQQGPGGSAAAAAGGYGPGGQGPGQQGPGSSAAAAAGPGGYGPGGQGPSASAAAAAGPGSGQQGPGASAAAAAGGYGPGGQGPGQQGPGSSAAAAAGGYGSGPGQQGPYGSAAAAAGPGSGGYGQGPYGPGASAAAAAGPGGYGPGGQGPSASAAAAAGSGQQGPGGYGPYASAAAAAGGYGSGPGQQGPYGPGGSAAAAAGSGQQGPGQQGPYASAAAAAGPGGQGPYGPGSSAAAAAGGYGYGPGGQGPYGPGASAAAAAGGNGPGSGGYGPGQQGPGGSAAAAAGPGGQGPYGPGASAAAAAGGYGPGGQGPGGYGPGSSAAAAAGPGGQGPYGPGSSAAAAAGGYGPGQQGPYGPGGSAAAAAGGYQQGPGGQGPYGPGASAAAAAGPGGQGPYGPGASAAAAAGPGGYGPGGQGPSASAAAAAGGYGSGPGGYGPYGPGGSAAAAAGPGSGQQGQGPYGPGASAAAAAGGYGPGQQGPYGPGGSAAAAAGPGSGGYGPGASAAAAAGGNGPGSGGYGPGQQGPGGSAAAAAGGYQQGPGGQGPYGPGASAAAAAGPGSGQQGPGAS

SEQ ID NO: 17 - protein, 590 aa, Artificial Sequence
  Met-PRT399
MGPGGQGPYGPGASAAAAAGGNGPGSGQQGPGGSGGYGPGGQGPGQQGPGSSAAAAAGPGGYGPGGQGPSASAAAAAGPGSGQQGPGASGGYGPGGQGPGQQGPGSSAAAAAGGYGSGPGQQGPYGSAAAAAGPGSGGYGQGPYGPGASGPGGYGPGGQGPSASAAAAAGSGQQGPGGYGPYASAAAAAGGYGSGPGQQGPYGPGGSGSGQQGPGQQGPYASAAAAAGPGGQGPYGPGSSAAAAAGGYGYGPGGQGPYGPGASGGNGPGSGGYGPGQQGPGGSAAAAAGPGGQGPYGPGASAAAAAGGYGPGGQGPGGYGPGSSGPGGQGPYGPGSSAAAAAGGYGPGQQGPYGPGGSAAAAAGGYQQGPGGQGPYGPGASGPGGQGPYGPGASAAAAAGPGGYGPGGQGPSASAAAAAGGYGSGPGGYGPYGPGGSGPGSGQQGQGPYGPGASAAAAAGGYGPGQQGPYGPGGSAAAAAGPGSGGYGPGASGGNGPGSGGYGPGQQGPGGSAAAAAGGYQQGPGGQGPYGPGASAAAAAGGYGSGPGQQGPYGPGGSGSGQQGPGQQGPYASAAAAAGPGSGQQGPGAS

SEQ ID NO: 18 - protein, 601 aa, Artificial Sequence
  PRT399
MHHHHHHSSGSSGPGGQGPYGPGASAAAAAGGNGPGSGQQGPGGSGGYGPGGQGPGQQGPGSSAAAAAGPGGYGPGGQGPSASAAAAAGPGSGQQGPGASGGYGPGGQGPGQQGPGSSAAAAAGGYGSGPGQQGPYGSAAAAAGPGSGGYGQGPYGPGASGPGGYGPGGQGPSASAAAAAGSGQQGPGGYGPYASAAAAAGGYGSGPGQQGPYGPGGSGSGQQGPGQQGPYASAAAAAGPGGQGPYGPGSSAAAAAGGYGYGPGGQGPYGPGASGGNGPGSGGYGPGQQGPGGSAAAAAGPGGQGPYGPGASAAAAAGGYGPGGQGPGGYGPGSSGPGGQGPYGPGSSAAAAAGGYGPGQQGPYGPGGSAAAAAGGYQQGPGGQGPYGPGASGPGGQGPYGPGASAAAAAGPGGYGPGGQGPSASAAAAAGGYGSGPGGYGPYGPGGSGPGSGQQGQGPYGPGASAAAAAGGYGPGQQGPYGPGGSAAAAAGPGSGGYGPGASGGNGPGSGGYGPGQQGPGGSAAAAAGGYQQGPGGQGPYGPGASAAAAAGGYGSGPGQQGPYGPGGSGSGQQGPGQQGPYASAAAAAGPGSGQQGPGAS

SEQ ID NO: 19 - protein, 612 aa, Artificial Sequence
  Met-PRT720
MGPGQQGPYGPGASAAAAAGQNGPGSGQQGPGQSGQYGPGQQGPGQQGPGSSAAAAAGPGQYVLIGPGQQVLIGPSASAAAAAGPGSGQQGPGASGQYGPGQQGPGQQGPGSSAAAAAGSYGSVLIGPGQQVLIGPYGSAAAAAGPGSGQYGQGPYGPGASGPGQYGPGQQGPSASAAAAAGSGQQVLIGPGQYVLIGPYASAAAAAGQYGSGPGQQGPYGPGQSGSGQQGPGQQGPYASAAAAAGPGQQVLIGPYVLIGPGSSAAAAAGQYGYGPGQQGPYGPGASGQNGPGSGQYGPGQQGPGQSAAAAAGPGQQVLIGPYVLIGPGASAAAAAGQYGPGQQGPGQYGPGSSGPGQQGPYGPGSSAAAAAGSYGPGQQVLIGPYVLIGPGPSAAAAAGQYQQGPGQQGPYGPGASGPGQQGPYGPGASAAAAAGPGQYVLIGPGQQVLIGPSASAAAAAGQYGSGPGQYGPYGPGQSGPGSGQQGQGPYGPGASAAAAAGSYGPGQQVLIGPYVLIGPGPSAAAAAGPGSGQYGPGASGQNGPGSGQYGPGQQGPGQSAAAAAGQYQQVLIGPGQQGPYVLIGPGASAAAAAGPGSGQQVLIGPGASVLI

SEQ ID NO: 20 - protein, 592 aa, Artificial Sequence
  Met-PRT665
MGPGQQGPYGPGASAAAAAAAGSNGPGSGQQGPGQSGQYGPGQQGPGQQGPGSSAAAAAAAGPGQYVLIGPGQQGPSASAAAAAAAGPGSGQQGPGASGQYGPGQQGPGQQGPGSSAAAAAAAGSYGSVLIGPGQQGPYGSAAAAAAAGPGSGQYGQGPYGPGASGPGQYGPGQQGPSASAAAAAAAGSGQQVLIGPGQYGPYASAAAAAAAGSYGSGPGQQGPYGPGQSGSGQQGPGQQGPYASAAAAAAAGPGQQVLIGPYGPGSSAAAAAAAGSYGYGPGQQGPYGPGASGQNGPGSGQYGPGQQGPGPSAAAAAAAGPGQQVLIGPYGPGASAAAAAAAGSYGPGQQGPGQYGPGSSGPGQQGPYGPGSSAAAAAAAGSYGPGQQVLIGPYGPGPSAAAAAAAGSYQQGPGQQGPYGPGASGPGQQGPYGPGASAAAAAAAGPGQYVLIGPGQQGPSASAAAAAAAGSYGSGPGQYGPYGPGQSGPGSGQQGQGPYGPGASAAAAAAAGSYGPGQQVLIGPYGPGPSAAAAAAAGPGSGQYGPGASGQNGPGSGQYGPGQQGPGPSAAAAAAAGPGSGQQGPGASVLI

SEQ ID NO: 21 - protein, 619 aa, Artificial Sequence
  Met-PRT666
MGPGQQGPYGPGASAAAAAAAGSNGPGSGQQGPGQSGQYGPGQQGPGQQGPGSSAAAAAAAGPGQYVLIGPGQQVLIGPSASAAAAAAAGPGSGQQGPGASGQYGPGQQGPGQQGPGSSAAAAAAAGSYGSVLIGPGQQVLIGPYGSAAAAAAAGPGSGQYGQGPYGPGASGPGQYGPGQQGPSASAAAAAAAGSGQQVLIGPGQYVLIGPYASAAAAAAAGSYGSGPGQQGPYGPGQSGSGQQGPGQQGPYASAAAAAAAGPGQQVLIGPYVLIGPGSSAAAAAAAGSYGYGPGQQGPYGPGASGQNGPGSGQYGPGQQGPGPSAAAAAAAGPGQQVLIGPYVLIGPGASAAAAAAAGSYGPGQQGPGQYGPGSSGPGQQGPYGPGSSAAAAAAAGSYGPGQQVLIGPYVLIGPGPSAAAAAAAGSYQQGPGQQGPYGPGASGPGQQGPYGPGASAAAAAAAGPGQYVLIGPGQQVLIGPSASAAAAAAAGSYGSGPGQYGPYGPGQSGPGSGQQGQGPYGPGASAAAAAAAGSYGPGQQVLIGPYVLIGPGPSAAAAAAAGPGSGQYGPGASGQNGPGSGQYGPGQQGPGPSAAAAAAAGPGSGQQVLIGPGASVLI

SEQ ID NO: 22 - protein, 623 aa, Artificial Sequence
  PRT720
MHHHHHHSSGSSGPGQQGPYGPGASAAAAAGQNGPGSGQQGPGQSGQYGPGQQGPGQQGPGSSAAAAAGPGQYVLIGPGQQVLIGPSASAAAAAGPGSGQQGPGASGQYGPGQQGPGQQGPGSSAAAAAGSYGSVLIGPGQQVLIGPYGSAAAAAGPGSGQYGQGPYGPGASGPGQYGPGQQGPSASAAAAAGSGQQVLIGPGQYVLIGPYASAAAAAGQYGSGPGQQGPYGPGQSGSGQQGPGQQGPYASAAAAAGPGQQVLIGPYVLIGPGSSAAAAAGQYGYGPGQQGPYGPGASGQNGPGSGQYGPGQQGPGQSAAAAAGPGQQVLIGPYVLIGPGASAAAAAGQYGPGQQGPGQYGPGSSGPGQQGPYGPGSSAAAAAGSYGPGQQVLIGPYVLIGPGPSAAAAAGQYQQGPGQQGPYGPGASGPGQQGPYGPGASAAAAAGPGQYVLIGPGQQVLIGPSASAAAAAGQYGSGPGQYGPYGPGQSGPGSGQQGQGPYGPGASAAAAAGSYGPGQQVLIGPYVLIGPGPSAAAAAGPGSGQYGPGASGQNGPGSGQYGPGQQGPGQSAAAAAGQYQQVLIGPGQQGPYVLIGPGASAAAAAGPGSGQQVLIGPGASVLI

SEQ ID NO: 23 - protein, 603 aa, Artificial Sequence
  PRT665
MHHHHHHSSGSSGPGQQGPYGPGASAAAAAAAGSNGPGSGQQGPGQSGQYGPGQQGPGQQGPGSSAAAAAAAGPGQYVLIGPGQQGPSASAAAAAAAGPGSGQQGPGASGQYGPGQQGPGQQGPGSSAAAAAAAGSYGSVLIGPGQQGPYGSAAAAAAAGPGSGQYGQGPYGPGASGPGQYGPGQQGPSASAAAAAAAGSGQQVLIGPGQYGPYASAAAAAAAGSYGSGPGQQGPYGPGQSGSGQQGPGQQGPYASAAAAAAAGPGQQVLIGPYGPGSSAAAAAAAGSYGYGPGQQGPYGPGASGQNGPGSGQYGPGQQGPGPSAAAAAAAGPGQQVLIGPYGPGASAAAAAAAGSYGPGQQGPGQYGPGSSGPGQQGPYGPGSSAAAAAAAGSYGPGQQVLIGPYGPGPSAAAAAAAGSYQQGPGQQGPYGPGASGPGQQGPYGPGASAAAAAAAGPGQYVLIGPGQQGPSASAAAAAAAGSYGSGPGQYGPYGPGQSGPGSGQQGQGPYGPGASAAAAAAAGSYGPGQQVLIGPYGPGPSAAAAAAAGPGSGQYGPGASGQNGPGSGQYGPGQQGPGPSAAAAAAAGPGSGQQGPGASVLI

SEQ ID NO: 24 - protein, 630 aa, Artificial Sequence
  PRT666
MHHHHHHSSGSSGPGQQGPYGPGASAAAAAAAGSNGPGSGQQGPGQSGQYGPGQQGPGQQGPGSSAAAAAAAGPGQYVLIGPGQQVLIGPSASAAAAAAAGPGSGQQGPGASGQYGPGQQGPGQQGPGSSAAAAAAAGSYGSVLIGPGQQVLIGPYGSAAAAAAAGPGSGQYGQGPYGPGASGPGQYGPGQQGPSASAAAAAAAGSGQQVLIGPGQYVLIGPYASAAAAAAAGSYGSGPGQQGPYGPGQSGSGQQGPGQQGPYASAAAAAAAGPGQQVLIGPYVLIGPGSSAAAAAAAGSYGYGPGQQGPYGPGASGQNGPGSGQYGPGQQGPGPSAAAAAAAGPGQQVLIGPYVLIGPGASAAAAAAAGSYGPGQQGPGQYGPGSSGPGQQGPYGPGSSAAAAAAAGSYGPGQQVLIGPYVLIGPGPSAAAAAAAGSYQQGPGQQGPYGPGASGPGQQGPYGPGASAAAAAAAGPGQYVLIGPGQQVLIGPSASAAAAAAAGSYGSGPGQYGPYGPGQSGPGSGQQGQGPYGPGASAAAAAAAGSYGPGQQVLIGPYVLIGPGPSAAAAAAAGPGSGQYGPGASGQNGPGSGQYGPGQQGPGPSAAAAAAAGPGSGQQVLIGPGASVLI

SEQ ID NO: 25 - protein, 593 aa, Artificial Sequence
  Met-PRT888
MGSSGPGVLGPYGPGASAAAAAGQNGPGSGVLGPGQSGQYGPGVLGPGVLGPGSSAAAAAGPGQYGPGVLGPSASAAAAAGPGSGVLGPGASGQYGPGVLGPGVLGPGSSAAAAAGQYGSGPGVLGPYGSAAAAAGPGSGQYGQGPYGPGASGPGQYGPGVLGPSASAAAAAGSGVLGPGQYGPYASAAAAAGQYGSGPGVLGPYGPGQSGSGVLGPGVLGPYASAAAAAGPGVLGPYGPGSSAAAAAGQYGYGPGVLGPYGPGASGQNGPGSGQYGPGVLGPGQSAAAAAGPGVLGPYGPGASAAAAAGQYGPGVLGPGQYGPGSSGPGVLGPYGPGSSAAAAAGQYGPGVLGPYGPGQSAAAAAGQYVLGPGVLGPYGPGASGPGVLGPYGPGASAAAAAGPGQYGPGVLGPSASAAAAAGQYGSGPGQYGPYGPGQSGPGSGVLGQGPYGPGASAAAAAGQYGPGVLGPYGPGQSAAAAAGPGSGQYGPGASGQNGPGSGQYGPGVLGPGQSAAAAAGQYVLGPGVLGPYGPGASAAAAAGQYGSGPGVLGPYGPGQSGSGVLGPGVLGPYASAAAAAGPGSGVLGPGAS

SEQ ID NO: 26 - protein, 590 aa, Artificial Sequence
  Met-PRT965
MGPGTSGPYGPGASAAAAAGANGPGSGTSGPGASGAYGPGTSGPGTSGPGSSAAAAAGPGAYGPGTSGPSASAAAAAGPGSGTSGPGASGAYGPGTSGPGTSGPGSSAAAAAGAYGSGPGTSGPYGSAAAAAGPGSGAYGAGPYGPGASGPGAYGPGTSGPSASAAAAAGSGTSGPGAYGPYASAAAAAGAYGSGPGTSGPYGPGASGSGTSGPGTSGPYASAAAAAGPGTSGPYGPGSSAAAAAGAYGYGPGTSGPYGPGASGANGPGSGAYGPGTSGPGASAAAAAGPGTSGPYGPGASAAAAAGAYGPGTSGPGAYGPGSSGPGTSGPYGPGSSAAAAAGAYGPGTSGPYGPGASAAAAAGAYTSGPGTSGPYGPGASGPGTSGPYGPGASAAAAAGPGAYGPGTSGPSASAAAAAGAYGSGPGAYGPYGPGASGPGSGTSGAGPYGPGASAAAAAGAYGPGTSGPYGPGASAAAAAGPGSGAYGPGASGANGPGSGAYGPGTSGPGASAAAAAGAYTSGPGTSGPYGPGASAAAAAGAYGSGPGTSGPYGPGASGSGTSGPGTSGPYASAAAAAGPGSGTSGPGAS

SEQ ID NO: 27 - protein, 593 aa, Artificial Sequence
  Met-PRT889
MGSSGPGVLGPYGPGASAAAAAGINGPGSGVLGPGISGIYGPGVLGPGVLGPGSSAAAAAGPGIYGPGVLGPSASAAAAAGPGSGVLGPGASGIYGPGVLGPGVLGPGSSAAAAAGIYGSGPGVLGPYGSAAAAAGPGSGIYGIGPYGPGASGPGIYGPGVLGPSASAAAAAGSGVLGPGIYGPYASAAAAAGIYGSGPGVLGPYGPGISGSGVLGPGVLGPYASAAAAAGPGVLGPYGPGSSAAAAAGIYGYGPGVLGPYGPGASGINGPGSGIYGPGVLGPGISAAAAAGPGVLGPYGPGASAAAAAGIYGPGVLGPGIYGPGSSGPGVLGPYGPGSSAAAAAGIYGPGVLGPYGPGISAAAAAGIYVLGPGVLGPYGPGASGPGVLGPYGPGASAAAAAGPGIYGPGVLGPSASAAAAAGIYGSGPGIYGPYGPGISGPGSGVLGIGPYGPGASAAAAAGIYGPGVLGPYGPGISAAAAAGPGSGIYGPGASGINGPGSGIYGPGVLGPGISAAAAAGIYVLGPGVLGPYGPGASAAAAAGIYGSGPGVLGPYGPGISGSGVLGPGVLGPYASAAAAAGPGSGVLGPGAS

SEQ ID NO: 28 - protein, 590 aa, Artificial Sequence
  Met-PRT916
MGPGVIGPYGPGASAAAAAGLNGPGSGVIGPGLSGLYGPGVIGPGVIGPGSSAAAAAGPGLYGPGVIGPSASAAAAAGPGSGVIGPGASGLYGPGVIGPGVIGPGSSAAAAAGLYGSGPGVIGPYGSAAAAAGPGSGLYGLGPYGPGASGPGLYGPGVIGPSASAAAAAGSGVIGPGLYGPYASAAAAAGLYGSGPGVIGPYGPGLSGSGVIGPGVIGPYASAAAAAGPGVIGPYGPGSSAAAAAGLYGYGPGVIGPYGPGASGLNGPGSGLYGPGVIGPGLSAAAAAGPGVIGPYGPGASAAAAAGLYGPGVIGPGLYGPGSSGPGVIGPYGPGSSAAAAAGLYGPGVIGPYGPGLSAAAAAGLYVIGPGVIGPYGPGASGPGVIGPYGPGASAAAAAGPGLYGPGVIGPSASAAAAAGLYGSGPGLYGPYGPGLSGPGSGVIGLGPYGPGASAAAAAGLYGPGVIGPYGPGLSAAAAAGPGSGLYGPGASGLNGPGSGLYGPGVIGPGLSAAAAAGLYVIGPGVIGPYGPGASAAAAAGLYGSGPGVIGPYGPGLSGSGVIGPGVIGPYASAAAAAGPGSGVIGPGAS

SEQ ID NO: 29 - protein, 590 aa, Artificial Sequence
  Met-PRT918
MGPGVFGPYGPGASAAAAAGINGPGSGVFGPGISGIYGPGVFGPGVFGPGSSAAAAAGPGIYGPGVFGPSASAAAAAGPGSGVFGPGASGIYGPGVFGPGVFGPGSSAAAAAGIYGSGPGVFGPYGSAAAAAGPGSGIYGIGPYGPGASGPGIYGPGVFGPSASAAAAAGSGVFGPGIYGPYASAAAAAGIYGSGPGVFGPYGPGISGSGVFGPGVFGPYASAAAAAGPGVFGPYGPGSSAAAAAGIYGYGPGVFGPYGPGASGINGPGSGIYGPGVFGPGISAAAAAGPGVFGPYGPGASAAAAAGIYGPGVFGPGIYGPGSSGPGVFGPYGPGSSAAAAAGIYGPGVFGPYGPGISAAAAAGIYVFGPGVFGPYGPGASGPGVFGPYGPGASAAAAAGPGIYGPGVFGPSASAAAAAGIYGSGPGIYGPYGPGISGPGSGVFGIGPYGPGASAAAAAGIYGPGVFGPYGPGISAAAAAGPGSGIYGPGASGINGPGSGIYGPGVFGPGISAAAAAGIYVFGPGVFGPYGPGASAAAAAGIYGSGPGVFGPYGPGISGSGVFGPGVFGPYASAAAAAGPGSGVFGPGAS

SEQ ID NO: 30 - protein, 565 aa, Artificial Sequence
  Met-PRT699
MGPGVLGPYGPGASAAAAAAAGSNGPGSGVLGPGQSGQYGPGVLGPGVLGPGSSAAAAAAAGPGQYGPGVLGPSASAAAAAAAGPGSGVLGPGASGQYGPGVLGPGVLGPGSSAAAAAAAGSYGSGPGVLGPYGSAAAAAAAGPGSGQYGQGPYGPGASGPGQYGPGVLGPSASAAAAAAAGSGVLGPGQYGPYASAAAAAAAGSYGSGPGVLGPYGPGQSGSGVLGPGVLGPYASAAAAAAAGPGVLGPYGPGSSAAAAAAAGSYGYGPGVLGPYGPGASGQNGPGSGQYGPGVLGPGPSAAAAAAAGPGVLGPYGPGASAAAAAAAGSYGPGVLGPGQYGPGSSGPGVLGPYGPGSSAAAAAAAGSYGPGVLGPYGPGPSAAAAAAAGSYVLGPGVLGPYGPGASGPGVLGPYGPGASAAAAAAAGPGQYGPGVLGPSASAAAAAAAGSYGSGPGQYGPYGPGQSGPGSGVLGQGPYGPGASAAAAAAAGSYGPGVLGPYGPGPSAAAAAAAGPGSGQYGPGASGQNGPGSGQYGPGVLGPGPSAAAAAAAGPGSGVLGPGAS

SEQ ID NO: 31 - protein, 565 aa, Artificial Sequence
  Met-PRT698
MGPGVLGPYGPGASAAAAAAAGSNGPGSGVLGPGISGIYGPGVLGPGVLGPGSSAAAAAAAGPGIYGPGVLGPSASAAAAAAAGPGSGVLGPGASGIYGPGVLGPGVLGPGSSAAAAAAAGSYGSGPGVLGPYGSAAAAAAAGPGSGIYGIGPYGPGASGPGIYGPGVLGPSASAAAAAAAGSGVLGPGIYGPYASAAAAAAAGSYGSGPGVLGPYGPGISGSGVLGPGVLGPYASAAAAAAAGPGVLGPYGPGSSAAAAAAAGSYGYGPGVLGPYGPGASGINGPGSGIYGPGVLGPGPSAAAAAAAGPGVLGPYGPGASAAAAAAAGSYGPGVLGPGIYGPGSSGPGVLGPYGPGSSAAAAAAAGSYGPGVLGPYGPGPSAAAAAAAGSYVLGPGVLGPYGPGASGPGVLGPYGPGASAAAAAAAGPGIYGPGVLGPSASAAAAAAAGSYGSGPGIYGPYGPGISGPGSGVLGIGPYGPGASAAAAAAAGSYGPGVLGPYGPGPSAAAAAAAGPGSGIYGPGASGINGPGSGIYGPGVLGPGPSAAAAAAAGPGSGVLGPGAS

SEQ ID NO: 32 - protein, 1179 aa, Artificial Sequence
  Met-PRT966
MGPGVFGPYGPGASAAAAAGINGPGSGVFGPGISGIYGPGVFGPGVFGPGSSAAAAAGPGIYGPGVFGPSASAAAAAGPGSGVFGPGASGIYGPGVFGPGVFGPGSSAAAAAGIYGSGPGVFGPYGSAAAAAGPGSGIYGIGPYGPGASGPGIYGPGVFGPSASAAAAAGSGVFGPGIYGPYASAAAAAGIYGSGPGVFGPYGPGISGSGVFGPGVFGPYASAAAAAGPGVFGPYGPGSSAAAAAGIYGYGPGVFGPYGPGASGINGPGSGIYGPGVFGPGISAAAAAGPGVFGPYGPGASAAAAAGIYGPGVFGPGIYGPGSSGPGVFGPYGPGSSAAAAAGIYGPGVFGPYGPGISAAAAAGIYVFGPGVFGPYGPGASGPGVFGPYGPGASAAAAAGPGIYGPGVFGPSASAAAAAGIYGSGPGIYGPYGPGISGPGSGVFGIGPYGPGASAAAAAGIYGPGVFGPYGPGISAAAAAGPGSGIYGPGASGINGPGSGIYGPGVFGPGISAAAAAGIYVFGPGVFGPYGPGASAAAAAGIYGSGPGVFGPYGPGISGSGVFGPGVFGPYASAAAAAGPGSGVFGPGASGPGVFGPYGPGASAAAAAGINGPGSGVFGPGISGIYGPGVFGPGVFGPGSSAAAAAGPGIYGPGVFGPSASAAAAAGPGSGVFGPGASGIYGPGVFGPGVFGPGSSAAAAAGIYGSGPGVFGPYGSAAAAAGPGSGIYGIGPYGPGASGPGIYGPGVFGPSASAAAAAGSGVFGPGIYGPYASAAAAAGIYGSGPGVFGPYGPGISGSGVFGPGVFGPYASAAAAAGPGVFGPYGPGSSAAAAAGIYGYGPGVFGPYGPGASGINGPGSGIYGPGVFGPGISAAAAAGPGVFGPYGPGASAAAAAGIYGPGVFGPGIYGPGSSGPGVFGPYGPGSSAAAAAGIYGPGVFGPYGPGISAAAAAGIYVFGPGVFGPYGPGASGPGVFGPYGPGASAAAAAGPGIYGPGVFGPSASAAAAAGIYGSGPGIYGPYGPGISGPGSGVFGIGPYGPGASAAAAAGIYGPGVFGPYGPGISAAAAAGPGSGIYGPGASGINGPGSGIYGPGVFGPGISAAAAAGIYVFGPGVFGPYGPGASAAAAAGIYGSGPGVFGPYGPGISGSGVFGPGVFGPYASAAAAAGPGSGVFGPGAS

SEQ ID NO: 33 - protein, 601 aa, Artificial Sequence
  PRT888
MHHHHHHSSGSSGPGVLGPYGPGASAAAAAGQNGPGSGVLGPGQSGQYGPGVLGPGVLGPGSSAAAAAGPGQYGPGVLGPSASAAAAAGPGSGVLGPGASGQYGPGVLGPGVLGPGSSAAAAAGQYGSGPGVLGPYGSAAAAAGPGSGQYGQGPYGPGASGPGQYGPGVLGPSASAAAAAGSGVLGPGQYGPYASAAAAAGQYGSGPGVLGPYGPGQSGSGVLGPGVLGPYASAAAAAGPGVLGPYGPGSSAAAAAGQYGYGPGVLGPYGPGASGQNGPGSGQYGPGVLGPGQSAAAAAGPGVLGPYGPGASAAAAAGQYGPGVLGPGQYGPGSSGPGVLGPYGPGSSAAAAAGQYGPGVLGPYGPGQSAAAAAGQYVLGPGVLGPYGPGASGPGVLGPYGPGASAAAAAGPGQYGPGVLGPSASAAAAAGQYGSGPGQYGPYGPGQSGPGSGVLGQGPYGPGASAAAAAGQYGPGVLGPYGPGQSAAAAAGPGSGQYGPGASGQNGPGSGQYGPGVLGPGQSAAAAAGQYVLGPGVLGPYGPGASAAAAAGQYGSGPGVLGPYGPGQSGSGVLGPGVLGPYASAAAAAGPGSGVLGPGAS

SEQ ID NO: 34 - protein, 601 aa, Artificial Sequence
  PRT965
MHHHHHHSSGSSGPGTSGPYGPGASAAAAAGANGPGSGTSGPGASGAYGPGTSGPGTSGPGSSAAAAAGPGAYGPGTSGPSASAAAAAGPGSGTSGPGASGAYGPGTSGPGTSGPGSSAAAAAGAYGSGPGTSGPYGSAAAAAGPGSGAYGAGPYGPGASGPGAYGPGTSGPSASAAAAAGSGTSGPGAYGPYASAAAAAGAYGSGPGTSGPYGPGASGSGTSGPGTSGPYASAAAAAGPGTSGPYGPGSSAAAAAGAYGYGPGTSGPYGPGASGANGPGSGAYGPGTSGPGASAAAAAGPGTSGPYGPGASAAAAAGAYGPGTSGPGAYGPGSSGPGTSGPYGPGSSAAAAAGAYGPGTSGPYGPGASAAAAAGAYTSGPGTSGPYGPGASGPGTSGPYGPGASAAAAAGPGAYGPGTSGPSASAAAAAGAYGSGPGAYGPYGPGASGPGSGTSGAGPYGPGASAAAAAGAYGPGTSGPYGPGASAAAAAGPGSGAYGPGASGANGPGSGAYGPGTSGPGASAAAAAGAYTSGPGTSGPYGPGASAAAAAGAYGSGPGTSGPYGPGASGSGTSGPGTSGPYASAAAAAGPGSGTSGPGAS

SEQ ID NO: 35 - protein, 601 aa, Artificial Sequence
  PRT889
MHHHHHHSSGSSGPGVLGPYGPGASAAAAAGINGPGSGVLGPGISGIYGPGVLGPGVLGPGSSAAAAAGPGIYGPGVLGPSASAAAAAGPGSGVLGPGASGIYGPGVLGPGVLGPGSSAAAAAGIYGSGPGVLGPYGSAAAAAGPGSGIYGIGPYGPGASGPGIYGPGVLGPSASAAAAAGSGVLGPGIYGPYASAAAAAGIYGSGPGVLGPYGPGISGSGVLGPGVLGPYASAAAAAGPGVLGPYGPGSSAAAAAGIYGYGPGVLGPYGPGASGINGPGSGIYGPGVLGPGISAAAAAGPGVLGPYGPGASAAAAAGIYGPGVLGPGIYGPGSSGPGVLGPYGPGSSAAAAAGIYGPGVLGPYGPGISAAAAAGIYVLGPGVLGPYGPGASGPGVLGPYGPGASAAAAAGPGIYGPGVLGPSASAAAAAGIYGSGPGIYGPYGPGISGPGSGVLGIGPYGPGASAAAAAGIYGPGVLGPYGPGISAAAAAGPGSGIYGPGASGINGPGSGIYGPGVLGPGISAAAAAGIYVLGPGVLGPYGPGASAAAAAGIYGSGPGVLGPYGPGISGSGVLGPGVLGPYASAAAAAGPGSGVLGPGAS

SEQ ID NO: 36 - protein, 601 aa, Artificial Sequence
  PRT916
MHHHHHHSSGSSGPGVIGPYGPGASAAAAAGLNGPGSGVIGPGLSGLYGPGVIGPGVIGPGSSAAAAAGPGLYGPGVIGPSASAAAAAGPGSGVIGPGASGLYGPGVIGPGVIGPGSSAAAAAGLYGSGPGVIGPYGSAAAAAGPGSGLYGLGPYGPGASGPGLYGPGVIGPSASAAAAAGSGVIGPGLYGPYASAAAAAGLYGSGPGVIGPYGPGLSGSGVIGPGVIGPYASAAAAAGPGVIGPYGPGSSAAAAAGLYGYGPGVIGPYGPGASGLNGPGSGLYGPGVIGPGLSAAAAAGPGVIGPYGPGASAAAAAGLYGPGVIGPGLYGPGSSGPGVIGPYGPGSSAAAAAGLYGPGVIGPYGPGLSAAAAAGLYVIGPGVIGPYGPGASGPGVIGPYGPGASAAAAAGPGLYGPGVIGPSASAAAAAGLYGSGPGLYGPYGPGLSGPGSGVIGLGPYGPGASAAAAAGLYGPGVIGPYGPGLSAAAAAGPGSGLYGPGASGLNGPGSGLYGPGVIGPGLSAAAAAGLYVIGPGVIGPYGPGASAAAAAGLYGSGPGVIGPYGPGLSGSGVIGPGVIGPYASAAAAAGPGSGVIGPGAS

SEQ ID NO: 37 - protein, 601 aa, Artificial Sequence
  PRT918
MHHHHHHSSGSSGPGVFGPYGPGASAAAAAGINGPGSGVFGPGISGIYGPGVFGPGVFGPGSSAAAAAGPGIYGPGVFGPSASAAAAAGPGSGVFGPGASGIYGPGVFGPGVFGPGSSAAAAAGIYGSGPGVFGPYGSAAAAAGPGSGIYGIGPYGPGASGPGIYGPGVFGPSASAAAAAGSGVFGPGIYGPYASAAAAAGIYGSGPGVFGPYGPGISGSGVFGPGVFGPYASAAAAAGPGVFGPYGPGSSAAAAAGIYGYGPGVFGPYGPGASGINGPGSGIYGPGVFGPGISAAAAAGPGVFGPYGPGASAAAAAGIYGPGVFGPGIYGPGSSGPGVFGPYGPGSSAAAAAGIYGPGVFGPYGPGISAAAAAGIYVFGPGVFGPYGPGASGPGVFGPYGPGASAAAAAGPGIYGPGVFGPSASAAAAAGIYGSGPGIYGPYGPGISGPGSGVFGIGPYGPGASAAAAAGIYGPGVFGPYGPGISAAAAAGPGSGIYGPGASGINGPGSGIYGPGVFGPGISAAAAAGIYVFGPGVFGPYGPGASAAAAAGIYGSGPGVFGPYGPGISGSGVFGPGVFGPYASAAAAAGPGSGVFGPGAS

SEQ ID NO: 38 - protein, 576 aa, Artificial Sequence
  PRT699
MHHHHHHSSGSSGPGVLGPYGPGASAAAAAAAGSNGPGSGVLGPGQSGQYGPGVLGPGVLGPGSSAAAAAAAGPGQYGPGVLGPSASAAAAAAAGPGSGVLGPGASGQYGPGVLGPGVLGPGSSAAAAAAAGSYGSGPGVLGPYGSAAAAAAAGPGSGQYGQGPYGPGASGPGQYGPGVLGPSASAAAAAAAGSGVLGPGQYGPYASAAAAAAAGSYGSGPGVLGPYGPGQSGSGVLGPGVLGPYASAAAAAAAGPGVLGPYGPGSSAAAAAAAGSYGYGPGVLGPYGPGASGQNGPGSGQYGPGVLGPGPSAAAAAAAGPGVLGPYGPGASAAAAAAAGSYGPGVLGPGQYGPGSSGPGVLGPYGPGSSAAAAAAAGSYGPGVLGPYGPGPSAAAAAAAGSYVLGPGVLGPYGPGASGPGVLGPYGPGASAAAAAAAGPGQYGPGVLGPSASAAAAAAAGSYGSGPGQYGPYGPGQSGPGSGVLGQGPYGPGASAAAAAAAGSYGPGVLGPYGPGPSAAAAAAAGPGSGQYGPGASGQNGPGSGQYGPGVLGPGPSAAAAAAAGPGSGVLGPGAS

SEQ ID NO: 39 - protein, 576 aa, Artificial Sequence
  PRT698
MHHHHHHSSGSSGPGVLGPYGPGASAAAAAAAGSNGPGSGVLGPGISGIYGPGVLGPGVLGPGSSAAAAAAAGPGIYGPGVLGPSASAAAAAAAGPGSGVLGPGASGIYGPGVLGPGVLGPGSSAAAAAAAGSYGSGPGVLGPYGSAAAAAAAGPGSGIYGIGPYGPGASGPGIYGPGVLGPSASAAAAAAAGSGVLGPGIYGPYASAAAAAAAGSYGSGPGVLGPYGPGISGSGVLGPGVLGPYASAAAAAAAGPGVLGPYGPGSSAAAAAAAGSYGYGPGVLGPYGPGASGINGPGSGIYGPGVLGPGPSAAAAAAAGPGVLGPYGPGASAAAAAAAGSYGPGVLGPGIYGPGSSGPGVLGPYGPGSSAAAAAAAGSYGPGVLGPYGPGPSAAAAAAAGSYVLGPGVLGPYGPGASGPGVLGPYGPGASAAAAAAAGPGIYGPGVLGPSASAAAAAAAGSYGSGPGIYGPYGPGISGPGSGVLGIGPYGPGASAAAAAAAGSYGPGVLGPYGPGPSAAAAAAAGPGSGIYGPGASGINGPGSGIYGPGVLGPGPSAAAAAAAGPGSGVLGPGAS

SEQ ID NO: 40 - protein, 1190 aa, Artificial Sequence
  PRT966
MHHHHHHSSGSSGPGVFGPYGPGASAAAAAGINGPGSGVFGPGISGIYGPGVFGPGVFGPGSSAAAAAGPGIYGPGVFGPSASAAAAAGPGSGVFGPGASGIYGPGVFGPGVFGPGSSAAAAAGIYGSGPGVFGPYGSAAAAAGPGSGIYGIGPYGPGASGPGIYGPGVFGPSASAAAAAGSGVFGPGIYGPYASAAAAAGIYGSGPGVFGPYGPGISGSGVFGPGVFGPYASAAAAAGPGVFGPYGPGSSAAAAAGIYGYGPGVFGPYGPGASGINGPGSGIYGPGVFGPGISAAAAAGPGVFGPYGPGASAAAAAGIYGPGVFGPGIYGPGSSGPGVFGPYGPGSSAAAAAGIYGPGVFGPYGPGISAAAAAGIYVFGPGVFGPYGPGASGPGVFGPYGPGASAAAAAGPGIYGPGVFGPSASAAAAAGIYGSGPGIYGPYGPGISGPGSGVFGIGPYGPGASAAAAAGIYGPGVFGPYGPGISAAAAAGPGSGIYGPGASGINGPGSGIYGPGVFGPGISAAAAAGIYVFGPGVFGPYGPGASAAAAAGIYGSGPGVFGPYGPGISGSGVFGPGVFGPYASAAAAAGPGSGVFGPGASGPGVFGPYGPGASAAAAAGINGPGSGVFGPGISGIYGPGVFGPGVFGPGSSAAAAAGPGIYGPGVFGPSASAAAAAGPGSGVFGPGASGIYGPGVFGPGVFGPGSSAAAAAGIYGSGPGVFGPYGSAAAAAGPGSGIYGIGPYGPGASGPGIYGPGVFGPSASAAAAAGSGVFGPGIYGPYASAAAAAGIYGSGPGVFGPYGPGISGSGVFGPGVFGPYASAAAAAGPGVFGPYGPGSSAAAAAGIYGYGPGVFGPYGPGASGINGPGSGIYGPGVFGPGISAAAAAGPGVFGPYGPGASAAAAAGIYGPGVFGPGIYGPGSSGPGVFGPYGPGSSAAAAAGIYGPGVFGPYGPGISAAAAAGIYVFGPGVFGPYGPGASGPGVFGPYGPGASAAAAAGPGIYGPGVFGPSASAAAAAGIYGSGPGIYGPYGPGISGPGSGVFGIGPYGPGASAAAAAGIYGPGVFGPYGPGISAAAAAGPGSGIYGPGASGINGPGSGIYGPGVFGPGISAAAAAGIYVFGPGVFGPYGPGASAAAAAGIYGSGPGVFGPYGPGISGSGVFGPGVFGPYASAAAAAGPGSGVFGPGAS

SEQ ID NO: 41 - protein, 590 aa, Artificial Sequence
  Met-PRT917
MGPGLIGPYGPGASAAAAAGVNGPGSGLIGPGVSGVYGPGLIGPGLIGPGSSAAAAAGPGVYGPGLIGPSASAAAAAGPGSGLIGPGASGVYGPGLIGPGLIGPGSSAAAAAGVYGSGPGLIGPYGSAAAAAGPGSGVYGVGPYGPGASGPGVYGPGLIGPSASAAAAAGSGLIGPGVYGPYASAAAAAGVYGSGPGLIGPYGPGVSGSGLIGPGLIGPYASAAAAAGPGLIGPYGPGSSAAAAAGVYGYGPGLIGPYGPGASGVNGPGSGVYGPGLIGPGVSAAAAAGPGLIGPYGPGASAAAAAGVYGPGLIGPGVYGPGSSGPGLIGPYGPGSSAAAAAGVYGPGLIGPYGPGVSAAAAAGVYLIGPGLIGPYGPGASGPGLIGPYGPGASAAAAAGPGVYGPGLIGPSASAAAAAGVYGSGPGVYGPYGPGVSGPGSGLIGVGPYGPGASAAAAAGVYGPGLIGPYGPGVSAAAAAGPGSGVYGPGASGVNGPGSGVYGPGLIGPGVSAAAAAGVYLIGPGLIGPYGPGASAAAAAGVYGSGPGLIGPYGPGVSGSGLIGPGLIGPYASAAAAAGPGSGLIGPGAS

SEQ ID NO: 42 - protein, 587 aa, Artificial Sequence
  Met-PRT1028
MGPGIFGPYGPGASAAAAAGTGPGSGIFGPGTSGTYGPGIFGPGIFGPGSSAAAAAGPGTYGPGIFGPSASAAAAAGPGSGIFGPGASGTYGPGIFGPGIFGPGSSAAAAAGTYGSGPGIFGPYGSAAAAAGPGSGTYGTGPYGPGASGPGTYGPGIFGPSASAAAAAGSGIFGPGTYGPYASAAAAAGTYGSGPGIFGPYGPGTSGSGIFGPGIFGPYASAAAAAGPGIFGPYGPGSSAAAAAGTYGYGPGIFGPYGPGASGTGPGSGTYGPGIFGPGTSAAAAAGPGIFGPYGPGASAAAAAGTYGPGIFGPGTYGPGSSGPGIFGPYGPGSSAAAAAGTYGPGIFGPYGPGTSAAAAAGTYIFGPGIFGPYGPGASGPGIFGPYGPGASAAAAAGPGTYGPGIFGPSASAAAAAGTYGSGPGTYGPYGPGTSGPGSGIFGTGPYGPGASAAAAAGTYGPGIFGPYGPGTSAAAAAGPGSGTYGPGASGTGPGSGTYGPGIFGPGTSAAAAAGTYIFGPGIFGPYGPGASAAAAAGTYGSGPGIFGPYGPGTSGSGIFGPGIFGPYASAAAAAGPGSGIFGPGAS

SEQ ID NO: 43 - protein, 601 aa, Artificial Sequence
  PRT917
MHHHHHHSSGSSGPGLIGPYGPGASAAAAAGVNGPGSGLIGPGVSGVYGPGLIGPGLIGPGSSAAAAAGPGVYGPGLIGPSASAAAAAGPGSGLIGPGASGVYGPGLIGPGLIGPGSSAAAAAGVYGSGPGLIGPYGSAAAAAGPGSGVYGVGPYGPGASGPGVYGPGLIGPSASAAAAAGSGLIGPGVYGPYASAAAAAGVYGSGPGLIGPYGPGVSGSGLIGPGLIGPYASAAAAAGPGLIGPYGPGSSAAAAAGVYGYGPGLIGPYGPGASGVNGPGSGVYGPGLIGPGVSAAAAAGPGLIGPYGPGASAAAAAGVYGPGLIGPGVYGPGSSGPGLIGPYGPGSSAAAAAGVYGPGLIGPYGPGVSAAAAAGVYLIGPGLIGPYGPGASGPGLIGPYGPGASAAAAAGPGVYGPGLIGPSASAAAAAGVYGSGPGVYGPYGPGVSGPGSGLIGVGPYGPGASAAAAAGVYGPGLIGPYGPGVSAAAAAGPGSGVYGPGASGVNGPGSGVYGPGLIGPGVSAAAAAGVYLIGPGLIGPYGPGASAAAAAGVYGSGPGLIGPYGPGVSGSGLIGPGLIGPYASAAAAAGPGSGLIGPGAS

SEQ ID NO: 44 - protein, 598 aa, Artificial Sequence
  PRT1028
MHHHHHHSSGSSGPGIFGPYGPGASAAAAAGTGPGSGIFGPGTSGTYGPGIFGPGIFGPGSSAAAAAGPGTYGPGIFGPSASAAAAAGPGSGIFGPGASGTYGPGIFGPGIFGPGSSAAAAAGTYGSGPGIFGPYGSAAAAAGPGSGTYGTGPYGPGASGPGTYGPGIFGPSASAAAAAGSGIFGPGTYGPYASAAAAAGTYGSGPGIFGPYGPGTSGSGIFGPGIFGPYASAAAAAGPGIFGPYGPGSSAAAAAGTYGYGPGIFGPYGPGASGTGPGSGTYGPGIFGPGTSAAAAAGPGIFGPYGPGASAAAAAGTYGPGIFGPGTYGPGSSGPGIFGPYGPGSSAAAAAGTYGPGIFGPYGPGTSAAAAAGTYIFGPGIFGPYGPGASGPGIFGPYGPGASAAAAAGPGTYGPGIFGPSASAAAAAGTYGSGPGTYGPYGPGTSGPGSGIFGTGPYGPGASAAAAAGTYGPGIFGPYGPGTSAAAAAGPGSGTYGPGASGTGPGSGTYGPGIFGPGTSAAAAAGTYIFGPGIFGPYGPGASAAAAAGTYGSGPGIFGPYGPGTSGSGIFGPGIFGPYASAAAAAGPGSGIFGPGAS